European Patent Application EP 4 451 276 A1, published October 23, 2024. Title: METHOD AND SYSTEM FOR STRATIFICATION OF SUBJECTS AS RESPONDERS AND NON-RESPONDERS FOR A THERAPY. Applicant: TATA CONSULTANCY SERVICES LIMITED. Application EP. The sequence listing filed with the application follows.

SEQUENCE LISTING (2 sequences)

SEQ ID NO: 1 - RNA, 1540 nt, Haemophilus parainfluenzae
  source 1..1540: mol_type = rRNA
gaattgaagagtttgatcatggctcagattgaacgctggcggcaggcttaacacatgcaagtcgaacggtaacatgaagaagcttgcttctttgatgacgagtggcggacgggtgagtaatgcttgggaatctagcttatggagggggataactacgggaaactgtagctaataccgcgtagtatcggaagatgaaagtgtgggaccttcgggccacatgccataggatgagcccaagtgggattaggtagttggtgaggtaaaggctcaccaagccgacgatctctagctggtctgagaggatgaccagccacactgggactgagacacggcccagactcctacgggaggcagcagtggggaatattgcgcaatgggggcaaccctgacgcagccatgccgcgtgaatgaagaaggccttcgggttgtaaagttctttcggtagcgaggaaggcatttagtttaatagactaggtgattgacgttaactacagaagaagcaccggctaactccgtgccagcagccgcggtaatacggagggtgcgagcgttaatcggaataactgggcgtaaagggcacgcaggcggtgacttaagtgaggtgtgaaagccccgggcttaacctgggaattgcatttcatactgggtcgctagagtactttagggaggggtagaattccacgtgtagcggtgaaatgcgtagagatgtggaggaataccgaaggcgaaggcagccccttgggaatgtactgacgctcatgtgcgaaagcgtggggagcaaacaggattagataccctggtagtccacgctgtaaacgatgtcgatttgggggttgagctttaagcttggcgcccgtagctaacgtgataaatcgaccgcctggggagtacggccgcaaggttaaaactcaaatgaattgacgggggcccgcacaagcggtggagcatgtggtttaattcgatgcaacgcgaagaaccttacctactcttgacatccagagaacattccagagatggattggtgccttcgggaactctgagacaggtgctgcatggctgtcgtcagctcgtgttgtgaaatgttgggttaagtcccgcaacgagcgcaacccttatcctttgttgccagcgattcggtcgggaactcaaaggagactgccggtgataaaccggaggaaggtggggatgacgtcaagtcatcatggcccttacgagtagggctacacacgtgctacaatggcgtatacagagggaagcgagagtgcgagctggagcgaatctcacaaagtacgtctaagtccggattggagtctgcaactcgactccatgaagtcggaatcgctagtaatcgcaaatcagaatgttgcggtgaatacgttcccgggccttgtacacaccgcccgtcacaccatgggagtgggttgtaccagaagtagatagcttaaccttcgggggggcgtttaccacggtatgattcatgactggggtgaagtcgtaacaaggtaaccgtaggggaacctgcggttggatcacctcctta

SEQ ID NO: 2 - RNA, 1527 nt, Rothia mucilaginosa
  source 1..1527: mol_type = rRNA
tcaacggagagtttgattctggctcaggacgaacgctggcggcgtgcttaacacatgcaagtcgaacgatgaagcctagcttgctaggtggattagtggcgaacgggtgagtaatacgtgagtaacctacctttaactctgggataagcccgggaaactgggtctaataccggatacgaccaatctccgcatggggtgttggtggaaagcgttatgtagtggttatagatgggctcacggcctatcagcttgttggtgaggtaacggctcaccaaggcgacgacgggtagccggcctgagagggtgaccggccacactgggactgagacacggcccagactcctacgggaggcagcagtggggaatattgcacaatgggcgcaagcctgatgcagcgacgccgcgtgagggatgacggccttcgggttgtaaacctctgttagcagggaagaagagagattgacggtacctgcagagaaagcgccggctaactacgtgccagcagccgcggtaatacgtagggcgcgagcgttgtccggaattattgggcgtaaagagcttgtaggcggtttgtcgcgtctgctgtgaaaggccggggcttaactccgtgtattgcagtgggtacgggcagactagagtgcagtaggggagactggaattcctggtgtagcggtggaatgcgcagatatcaggaggaacaccgatggcgaaggcaggtctctgggctgtaactgacgctgagaagcgaaagcatggggagcgaacaggattagataccctggtagtccatgccgtaaacgttgggcactaggtgtgggggacattccacgttttccgcgccgtagctaacgcattaagtgccccgcctggggagtacggccgcaaggctaaaactcaaagaaattgacgggggcccgcacaagcggcggagcatgcggattaattcgatgcaacgcgaagaaccttaccaaggcttgacatatactggaccgcatcagagatggtgtttcccttcggggctggtatacaggtggtgcatggttgtcgtcagctcgtgtcgtgagatgttgggttaagtcccgcaacgagcgcaaccctcgttctatgttgccagcacgttatggtggggactcataggagactgccggggtcaactcggaggaaggtggggatgacgtcaaatcatcatgccccttatgtcttgggcttcacgcatgctacaatggccggtacagagggttgcgatactgtgaggtggagctaatccctaaaagccggtctcagttcggattggggtctgcaactcgaccccatgaagtcggagtcgctagtaatcgcagatcagcaacgctgcggtgaatacgttcccgggccttgtacacaccgcccgtcaagtcacgaaagttggtaacacccaaagccggtggcctaaccttttggagggagccgtctaaggtgggattggcgattgggactaagtcgtaacaaggtagccgtaccggaaggtgcggctggatcacctccttt